European Patent Specification EP 3 513 656 B1, published July 5, 2023. Title: Agricultural and horticultural composition and method for cultivating plant. Applicant: Ajinomoto Co., Inc. The sequence listing filed with the application follows.

SEQUENCE LISTING (20 sequences)

SEQ ID NO: 1 - DNA, 20 bp, Artificial Sequence
  primer
caccattgggtgtgagcgat

SEQ ID NO: 2 - DNA, 20 bp, Artificial Sequence
  primer
gggcgacaaccttgatcttc

SEQ ID NO: 3 - DNA, 21 bp, Artificial Sequence
  primer
gtgttgactaaagatgctggg

SEQ ID NO: 4 - DNA, 22 bp, Artificial Sequence
  primer
ggtgaaagatcaccatcagcaa

SEQ ID NO: 5 - DNA, 20 bp, Artificial Sequence
  primer
cggttttgtccatggcaaag

SEQ ID NO: 6 - DNA, 21 bp, Artificial Sequence
  primer
accgtcaggatcaccgatatc

SEQ ID NO: 7 - DNA, 21 bp, Artificial Sequence
  primer
gttgatgccaaggcttgtact

SEQ ID NO: 8 - DNA, 20 bp, Artificial Sequence
  primer
caacatgtggtacatccggt

SEQ ID NO: 9 - DNA, 20 bp, Artificial Sequence
  primer
agggtcgtctagttcagcag

SEQ ID NO: 10 - DNA, 24 bp, Artificial Sequence
  primer
tgggcttgaactgtacatcgccaa

SEQ ID NO: 11 - DNA, 20 bp, Artificial Sequence
  primer
ttgggcttgttgagtgaagc

SEQ ID NO: 12 - DNA, 20 bp, Artificial Sequence
  primer
tgtcgttgccttgattcagg

SEQ ID NO: 13 - DNA, 23 bp, Artificial Sequence
  primer
ttgtgtttgccgctccagtggat

SEQ ID NO: 14 - DNA, 23 bp, Artificial Sequence
  primer
gcgccttcgattgaagccaagta

SEQ ID NO: 15 - DNA, 23 bp, Artificial Sequence
  primer
attattacattgagggacaaggc

SEQ ID NO: 16 - DNA, 23 bp, Artificial Sequence
  primer
tcatcagacaagactcaactgat

SEQ ID NO: 17 - DNA, 22 bp, Artificial Sequence
  primer
agacaagcactccctgaggacc

SEQ ID NO: 18 - DNA, 21 bp, Artificial Sequence
  primer
aactctggccaccatggctca

SEQ ID NO: 19 - DNA, 21 bp, Artificial Sequence
  primer
tgctttcgctgcagtgccaga

SEQ ID NO: 20 - DNA, 23 bp, Artificial Sequence
  primer
tgtctagcgcacaaccgtcaagg